European Patent Application EP 4 674 864 A1, published January 7, 2026. Title: 新型光敏感通道蛋白VR3.0及其用途. Applicant: 中眸医疗科技（武汉）有限公司. Application CN. The sequence listing filed with the application follows.

SEQUENCE LISTING (28 sequences)

SEQ ID NO: 1 - protein, 432 aa, synthetic construct
MPFCGGRPEDGWHHGSIHDMDYPLLGAMAAICSVFIGGSGAWMLYRLDLGLGYSCKPHHSGYAPEANSFSALSCLVSGTIYAAKTFDFFDGGGTPFSFNWYWYLDYVFTCPLILLDVLYTLEIPHKLRFVFAVIITLWCGVAAFVTPSAFRFGYYAVGCVWFVPFSFSLLRHVKQRYQVYPPKCQKLLFWACTIFFGFWPLFPILFLFSWLGTGHIDQQAFTIIHAFLDLFCKTVFGLIMTFFRLELEEHTEVLGLPLNEPKGKHLFLNDSAARHEKHLAGPGTESLTAASSKVKLQWIQKLLAEALTEASQLDLDTPTVVPAKVLSSATPERHLPLRQQKKEQQERGEKTMVYPQLSSAILLGSPAQEEEQGGGGGAKRERGRALVTPLPGDESPGGEHLPDSVQEHLLLAVGSHRMGQQNLRQLRERRRH

SEQ ID NO: 2 - protein, 38 aa, synthetic construct
MRPQILLLLALLTLGLANGTEGPNFYVPFSNKTGVVRS

SEQ ID NO: 3 - protein, 239 aa, synthetic construct
MVSKGEELFTGVVPILVELDGDVNGHKFSVSGEGEGDATYGKLTLKFICTTGKLPVPWPTLVTTFGYGLQCFARYPDHMKQHDFFKSAMPEGYVQERTIFFKDDGNYKTRAEVKFEGDTLVNRIELKGIDFKEDGNILGHKLEYNYNSHNVYIMADKQKNGIKVNFKIRHNIEDGSVQLADHYQQNTPIGDGPVLLPDNHYLSYQSALSKDPNEKRDHMVLLEFVTAAGITLGMDELYK

SEQ ID NO: 4 - protein, 20 aa, synthetic construct
KSRITSEGEYIPLDQIDINV

SEQ ID NO: 5 - protein, 7 aa, synthetic construct
FCYENEV

SEQ ID NO: 6 - DNA, 589 bp, synthetic construct
  source 1..589: mol_type = other DNA
aatcaacctctggattacaaaatttgtgaaagattgactggtattcttaactatgttgctccttttacgctatgtggatacgctgctttaatgcctttgtatcatgctattgcttcccgtatggctttcattttctcctccttgtataaatcctggttgctgtctctttatgaggagttgtggcccgttgtcaggcaacgtggcgtggtgtgcactgtgtttgctgacgcaacccccactggttggggcattgccaccacctgtcagctcctttccgggactttcgctttccccctccctattgccacggcggaactcatcgccgcctgccttgcccgctgctggacaggggctcggctgttgggcactgacaattccgtggtgttgtcggggaaatcatcgtcctttccttggctgctcgcctatgttgccacctggattctgcgcgggacgtccttctgctacgtcccttcggccctcaatccagcggaccttccttcccgcggcctgctgccggctctgcggcctcttccgcgtcttcgccttcgccctcagacgagtcggatctccctttgggccgcctccccgc

SEQ ID NO: 7 - DNA, 477 bp, synthetic construct
  source 1..477: mol_type = other DNA
gggtggcatccctgtgacccctccccagtgcctctcctggccctggaagttgccactccagtgcccaccagccttgtcctaataaaattaagttgcatcattttgtctgactaggtgtccttctataatattatggggtggaggggggtggtatggagcaaggggcaagttgggaagacaacctgtagggcctgcggggtctattgggaaccaagctggagtgcagtggcacaatcttggctcactgcaatctccgcctcctgggttcaagcgattctcctgcctcagcctcccgagttgttgggattccaggcatgcatgaccaggctcagctaatttttgtttttttggtagagacggggtttcaccatattggccaggctggtctccaactcctaatctcaggtgatctacccaccttggcctcccaaattgctgggattacaggcgtgaaccactgctcccttccctgtcctt

SEQ ID NO: 8 - protein, 427 aa, synthetic construct
GRPEDGWHHGSIHDMDYPLLGAMAAICSVFIGGSGAWMLYRLDLGLGYSCKPHHSGYAPEANSFSALSCLVSGTIYAAKTFDFFDGGGTPFSFNWYWYLDYVFTCPLILLDVLYTLEIPHKLRFVFAVIITLWCGVAAFVTPSAFRFGYYAVGCVWFVPFSFSLLRHVKQRYQVYPPKCQKLLFWACTIFFGFWPLFPILFLFSWLGTGHIDQQAFTIIHAFLDLFCKTVFGLIMTFFRLELEEHTEVLGLPLNEPKGKHLFLNDSAARHEKHLAGPGTESLTAASSKVKLQWIQKLLAEALTEASQLDLDTPTVVPAKVLSSATPERHLPLRQQKKEQQERGEKTMVYPQLSSAILLGSPAQEEEQGGGGGAKRERGRALVTPLPGDESPGGEHLPDSVQEHLLLAVGSHRMGQQNLRQLRERRRH

SEQ ID NO: 9 - protein, 422 aa, synthetic construct
GWHHGSIHDMDYPLLGAMAAICSVFIGGSGAWMLYRLDLGLGYSCKPHHSGYAPEANSFSALSCLVSGTIYAAKTFDFFDGGGTPFSFNWYWYLDYVFTCPLILLDVLYTLEIPHKLRFVFAVIITLWCGVAAFVTPSAFRFGYYAVGCVWFVPFSFSLLRHVKQRYQVYPPKCQKLLFWACTIFFGFWPLFPILFLFSWLGTGHIDQQAFTIIHAFLDLFCKTVFGLIMTFFRLELEEHTEVLGLPLNEPKGKHLFLNDSAARHEKHLAGPGTESLTAASSKVKLQWIQKLLAEALTEASQLDLDTPTVVPAKVLSSATPERHLPLRQQKKEQQERGEKTMVYPQLSSAILLGSPAQEEEQGGGGGAKRERGRALVTPLPGDESPGGEHLPDSVQEHLLLAVGSHRMGQQNLRQLRERRRH

SEQ ID NO: 10 - protein, 417 aa, synthetic construct
SIHDMDYPLLGAMAAICSVFIGGSGAWMLYRLDLGLGYSCKPHHSGYAPEANSFSALSCLVSGTIYAAKTFDFFDGGGTPFSFNWYWYLDYVFTCPLILLDVLYTLEIPHKLRFVFAVIITLWCGVAAFVTPSAFRFGYYAVGCVWFVPFSFSLLRHVKQRYQVYPPKCQKLLFWACTIFFGFWPLFPILFLFSWLGTGHIDQQAFTIIHAFLDLFCKTVFGLIMTFFRLELEEHTEVLGLPLNEPKGKHLFLNDSAARHEKHLAGPGTESLTAASSKVKLQWIQKLLAEALTEASQLDLDTPTVVPAKVLSSATPERHLPLRQQKKEQQERGEKTMVYPQLSSAILLGSPAQEEEQGGGGGAKRERGRALVTPLPGDESPGGEHLPDSVQEHLLLAVGSHRMGQQNLRQLRERRRH

SEQ ID NO: 11 - protein, 408 aa, synthetic construct
LGAMAAICSVFIGGSGAWMLYRLDLGLGYSCKPHHSGYAPEANSFSALSCLVSGTIYAAKTFDFFDGGGTPFSFNWYWYLDYVFTCPLILLDVLYTLEIPHKLRFVFAVIITLWCGVAAFVTPSAFRFGYYAVGCVWFVPFSFSLLRHVKQRYQVYPPKCQKLLFWACTIFFGFWPLFPILFLFSWLGTGHIDQQAFTIIHAFLDLFCKTVFGLIMTFFRLELEEHTEVLGLPLNEPKGKHLFLNDSAARHEKHLAGPGTESLTAASSKVKLQWIQKLLAEALTEASQLDLDTPTVVPAKVLSSATPERHLPLRQQKKEQQERGEKTMVYPQLSSAILLGSPAQEEEQGGGGGAKRERGRALVTPLPGDESPGGEHLPDSVQEHLLLAVGSHRMGQQNLRQLRERRRH

SEQ ID NO: 12 - protein, 330 aa, synthetic construct
MPFCGGRPEDGWHHGSIHDMDYPLLGAMAAICSVFIGGSGAWMLYRLDLGLGYSCKPHHSGYAPEANSFSALSCLVSGTIYAAKTFDFFDGGGTPFSFNWYWYLDYVFTCPLILLDVLYTLEIPHKLRFVFAVIITLWCGVAAFVTPSAFRFGYYAVGCVWFVPFSFSLLRHVKQRYQVYPPKCQKLLFWACTIFFGFWPLFPILFLFSWLGTGHIDQQAFTIIHAFLDLFCKTVFGLIMTFFRLELEEHTEVLGLPLNEPKGKHLFLNDSAARHEKHLAGPGTESLTAASSKVKLQWIQKLLAEALTEASQLDLDTPTVVPAKVLSSAT

SEQ ID NO: 13 - protein, 306 aa, synthetic construct
MPFCGGRPEDGWHHGSIHDMDYPLLGAMAAICSVFIGGSGAWMLYRLDLGLGYSCKPHHSGYAPEANSFSALSCLVSGTIYAAKTFDFFDGGGTPFSFNWYWYLDYVFTCPLILLDVLYTLEIPHKLRFVFAVIITLWCGVAAFVTPSAFRFGYYAVGCVWFVPFSFSLLRHVKQRYQVYPPKCQKLLFWACTIFFGFWPLFPILFLFSWLGTGHIDQQAFTIIHAFLDLFCKTVFGLIMTFFRLELEEHTEVLGLPLNEPKGKHLFLNDSAARHEKHLAGPGTESLTAASSKVKLQWIQKLLAEA

SEQ ID NO: 14 - protein, 283 aa, synthetic construct
MPFCGGRPEDGWHHGSIHDMDYPLLGAMAAICSVFIGGSGAWMLYRLDLGLGYSCKPHHSGYAPEANSFSALSCLVSGTIYAAKTFDFFDGGGTPFSFNWYWYLDYVFTCPLILLDVLYTLEIPHKLRFVFAVIITLWCGVAAFVTPSAFRFGYYAVGCVWFVPFSFSLLRHVKQRYQVYPPKCQKLLFWACTIFFGFWPLFPILFLFSWLGTGHIDQQAFTIIHAFLDLFCKTVFGLIMTFFRLELEEHTEVLGLPLNEPKGKHLFLNDSAARHEKHLAGPG

SEQ ID NO: 15 - protein, 273 aa, synthetic construct
MPFCGGRPEDGWHHGSIHDMDYPLLGAMAAICSVFIGGSGAWMLYRLDLGLGYSCKPHHSGYAPEANSFSALSCLVSGTIYAAKTFDFFDGGGTPFSFNWYWYLDYVFTCPLILLDVLYTLEIPHKLRFVFAVIITLWCGVAAFVTPSAFRFGYYAVGCVWFVPFSFSLLRHVKQRYQVYPPKCQKLLFWACTIFFGFWPLFPILFLFSWLGTGHIDQQAFTIIHAFLDLFCKTVFGLIMTFFRLELEEHTEVLGLPLNEPKGKHLFLNDSAA

SEQ ID NO: 16 - protein, 253 aa, synthetic construct
MPFCGGRPEDGWHHGSIHDMDYPLLGAMAAICSVFIGGSGAWMLYRLDLGLGYSCKPHHSGYAPEANSFSALSCLVSGTIYAAKTFDFFDGGGTPFSFNWYWYLDYVFTCPLILLDVLYTLEIPHKLRFVFAVIITLWCGVAAFVTPSAFRFGYYAVGCVWFVPFSFSLLRHVKQRYQVYPPKCQKLLFWACTIFFGFWPLFPILFLFSWLGTGHIDQQAFTIIHAFLDLFCKTVFGLIMTFFRLELEEHTEV

SEQ ID NO: 17 - protein, 242 aa, synthetic construct
MPFCGGRPEDGWHHGSIHDMDYPLLGAMAAICSVFIGGSGAWMLYRLDLGLGYSCKPHHSGYAPEANSFSALSCLVSGTIYAAKTFDFFDGGGTPFSFNWYWYLDYVFTCPLILLDVLYTLEIPHKLRFVFAVIITLWCGVAAFVTPSAFRFGYYAVGCVWFVPFSFSLLRHVKQRYQVYPPKCQKLLFWACTIFFGFWPLFPILFLFSWLGTGHIDQQAFTIIHAFLDLFCKTVFGLIMTF

SEQ ID NO: 18 - protein, 325 aa, synthetic construct
GRPEDGWHHGSIHDMDYPLLGAMAAICSVFIGGSGAWMLYRLDLGLGYSCKPHHSGYAPEANSFSALSCLVSGTIYAAKTFDFFDGGGTPFSFNWYWYLDYVFTCPLILLDVLYTLEIPHKLRFVFAVIITLWCGVAAFVTPSAFRFGYYAVGCVWFVPFSFSLLRHVKQRYQVYPPKCQKLLFWACTIFFGFWPLFPILFLFSWLGTGHIDQQAFTIIHAFLDLFCKTVFGLIMTFFRLELEEHTEVLGLPLNEPKGKHLFLNDSAARHEKHLAGPGTESLTAASSKVKLQWIQKLLAEALTEASQLDLDTPTVVPAKVLSSAT

SEQ ID NO: 19 - protein, 278 aa, synthetic construct
GRPEDGWHHGSIHDMDYPLLGAMAAICSVFIGGSGAWMLYRLDLGLGYSCKPHHSGYAPEANSFSALSCLVSGTIYAAKTFDFFDGGGTPFSFNWYWYLDYVFTCPLILLDVLYTLEIPHKLRFVFAVIITLWCGVAAFVTPSAFRFGYYAVGCVWFVPFSFSLLRHVKQRYQVYPPKCQKLLFWACTIFFGFWPLFPILFLFSWLGTGHIDQQAFTIIHAFLDLFCKTVFGLIMTFFRLELEEHTEVLGLPLNEPKGKHLFLNDSAARHEKHLAGPG

SEQ ID NO: 20 - protein, 268 aa, synthetic construct
GRPEDGWHHGSIHDMDYPLLGAMAAICSVFIGGSGAWMLYRLDLGLGYSCKPHHSGYAPEANSFSALSCLVSGTIYAAKTFDFFDGGGTPFSFNWYWYLDYVFTCPLILLDVLYTLEIPHKLRFVFAVIITLWCGVAAFVTPSAFRFGYYAVGCVWFVPFSFSLLRHVKQRYQVYPPKCQKLLFWACTIFFGFWPLFPILFLFSWLGTGHIDQQAFTIIHAFLDLFCKTVFGLIMTFFRLELEEHTEVLGLPLNEPKGKHLFLNDSAA

SEQ ID NO: 21 - protein, 273 aa, synthetic construct
GWHHGSIHDMDYPLLGAMAAICSVFIGGSGAWMLYRLDLGLGYSCKPHHSGYAPEANSFSALSCLVSGTIYAAKTFDFFDGGGTPFSFNWYWYLDYVFTCPLILLDVLYTLEIPHKLRFVFAVIITLWCGVAAFVTPSAFRFGYYAVGCVWFVPFSFSLLRHVKQRYQVYPPKCQKLLFWACTIFFGFWPLFPILFLFSWLGTGHIDQQAFTIIHAFLDLFCKTVFGLIMTFFRLELEEHTEVLGLPLNEPKGKHLFLNDSAARHEKHLAGPG

SEQ ID NO: 22 - protein, 263 aa, synthetic construct
GWHHGSIHDMDYPLLGAMAAICSVFIGGSGAWMLYRLDLGLGYSCKPHHSGYAPEANSFSALSCLVSGTIYAAKTFDFFDGGGTPFSFNWYWYLDYVFTCPLILLDVLYTLEIPHKLRFVFAVIITLWCGVAAFVTPSAFRFGYYAVGCVWFVPFSFSLLRHVKQRYQVYPPKCQKLLFWACTIFFGFWPLFPILFLFSWLGTGHIDQQAFTIIHAFLDLFCKTVFGLIMTFFRLELEEHTEVLGLPLNEPKGKHLFLNDSAA

SEQ ID NO: 23 - protein, 291 aa, synthetic construct
SIHDMDYPLLGAMAAICSVFIGGSGAWMLYRLDLGLGYSCKPHHSGYAPEANSFSALSCLVSGTIYAAKTFDFFDGGGTPFSFNWYWYLDYVFTCPLILLDVLYTLEIPHKLRFVFAVIITLWCGVAAFVTPSAFRFGYYAVGCVWFVPFSFSLLRHVKQRYQVYPPKCQKLLFWACTIFFGFWPLFPILFLFSWLGTGHIDQQAFTIIHAFLDLFCKTVFGLIMTFFRLELEEHTEVLGLPLNEPKGKHLFLNDSAARHEKHLAGPGTESLTAASSKVKLQWIQKLLAEA

SEQ ID NO: 24 - protein, 268 aa, synthetic construct
SIHDMDYPLLGAMAAICSVFIGGSGAWMLYRLDLGLGYSCKPHHSGYAPEANSFSALSCLVSGTIYAAKTFDFFDGGGTPFSFNWYWYLDYVFTCPLILLDVLYTLEIPHKLRFVFAVIITLWCGVAAFVTPSAFRFGYYAVGCVWFVPFSFSLLRHVKQRYQVYPPKCQKLLFWACTIFFGFWPLFPILFLFSWLGTGHIDQQAFTIIHAFLDLFCKTVFGLIMTFFRLELEEHTEVLGLPLNEPKGKHLFLNDSAARHEKHLAGPG

SEQ ID NO: 25 - protein, 258 aa, synthetic construct
SIHDMDYPLLGAMAAICSVFIGGSGAWMLYRLDLGLGYSCKPHHSGYAPEANSFSALSCLVSGTIYAAKTFDFFDGGGTPFSFNWYWYLDYVFTCPLILLDVLYTLEIPHKLRFVFAVIITLWCGVAAFVTPSAFRFGYYAVGCVWFVPFSFSLLRHVKQRYQVYPPKCQKLLFWACTIFFGFWPLFPILFLFSWLGTGHIDQQAFTIIHAFLDLFCKTVFGLIMTFFRLELEEHTEVLGLPLNEPKGKHLFLNDSAA

SEQ ID NO: 26 - protein, 227 aa, synthetic construct
SIHDMDYPLLGAMAAICSVFIGGSGAWMLYRLDLGLGYSCKPHHSGYAPEANSFSALSCLVSGTIYAAKTFDFFDGGGTPFSFNWYWYLDYVFTCPLILLDVLYTLEIPHKLRFVFAVIITLWCGVAAFVTPSAFRFGYYAVGCVWFVPFSFSLLRHVKQRYQVYPPKCQKLLFWACTIFFGFWPLFPILFLFSWLGTGHIDQQAFTIIHAFLDLFCKTVFGLIMTF

SEQ ID NO: 27 - protein, 305 aa, synthetic construct
MGFQLNPEYLNETILLDDCTPIYLNVGPLWEQKVARGTQWFGVILSLAFLIYYIWITYKATCGWEELYVCTIEFCKIVIELYFEFSPPAMIYQTNGEVTPWLRYAEWLLTCPVICIHLSNITGLNDDYSGRTMSLITSDLGGICMAVTSALSKGWLKWLFFVIGCCYGASTFYHAALIYIESYYTMPHGVCKNMVLAMAAVFFTSWFMFPGLFLAGPEGTNALSWAGSTIGHTVADLLSKNAWGMIGHFLRLEIHKHIIIHGDVRRPITVNTLGREVTVSCFVDKEEEDEDERISTKTYANRALE

SEQ ID NO: 28 - protein, 8 aa, synthetic construct
VDTSSRSR